European Patent Specification EP 3 469 077 B1, published May 13, 2026. Title: USE OF CPF1 ENDONUCLEASE FOR PLANT GENOME MODIFICATIONS. Applicant: Pioneer Hi-Bred International Inc. Cigan, Andrew  Mark Djukanovic, Vesna Young, Joshua  Keith. The sequence listing filed with the application follows.

SEQUENCE LISTING (50 sequences)

SEQ ID NO: 1 - DNA, 3924 bp, Acidaminococcus
  misc_feature (1)..(3924): Cpf1 Gene from Acidaminococcus sp. BV3L6
atgacccaatttgaaggttttaccaatttataccaagtttcgaagacccttcgttttgaactgattccccaaggaaaaacactcaaacatatccaggagcaagggttcattgaggaggataaagctcgcaatgaccattacaaagagttaaaaccaatcattgaccgcatctataagacttatgctgatcaatgtctccaactggtacagcttgactgggagaatctatctgcagccatagactcctatcgtaaggaaaaaaccgaagaaacacgaaatgcgctgattgaggagcaagcaacatatagaaatgcgattcatgactactttataggtcggacggataatctgacagatgccataaataagcgccatgctgaaatctataaaggactttttaaagctgaacttttcaatggaaaagttttaaagcaattagggaccgtaaccacgacagaacatgaaaatgctctactccgttcgtttgacaaatttacgacctatttttccggcttttatgaaaaccgaaaaaatgtctttagcgctgaagatatcagcacggcaattccccatcgaatcgtccaggacaatttccctaaatttaaggaaaactgccatatttttacaagattgataaccgcagttccttctttgcgggagcattttgaaaatgtcaaaaaggccattggaatctttgttagtacgtctattgaagaagtcttttcctttcccttttataatcaacttctaacccaaacgcaaattgatctttataatcaacttctcggcggcatatctagggaagcaggcacagaaaaaatcaagggacttaatgaagttctcaatctggctatccaaaaaaatgatgaaacagcccatataatcgcgtccctgccgcatcgttttattcctctttttaaacaaattctttccgatcgaaatacgttatcctttattttggaagaattcaaaagcgatgaggaagtcatccaatccttctgcaaatataaaaccctcttgagaaacgaaaatgtactggagactgcagaagcccttttcaatgaattaaattccattgatttgactcatatctttatttcccataaaaagttagaaaccatctcttcagcgctttgtgaccattgggataccttgcgcaatgcactttacgaaagacggatttctgaactcactggcaaaataacaaaaagtgccaaagaaaaagttcaaaggtcattaaaacatgaggatataaatctccaagaaattatttctgctgcaggaaaagaactatcagaagcattcaaacaaaaaacaagtgaaattctttcccatgcccatgctgcacttgaccagcctcttcccacaacattaaaaaaacaggaagaaaaagaaatcctcaaatcacagctcgattcgcttttaggcctttatcatcttcttgattggtttgctgtcgatgaaagcaatgaagtcgacccagaattctcagcacggctgacaggcattaaactagaaatggaaccaagcctttcgttttataataaagcaagaaattatgcgacaaaaaagccctattcggtggaaaaatttaaattgaattttcaaatgccaacccttgcctctggttgggatgtcaataaagaaaaaaataatggagctattttattcgtaaaaaatggtctctattaccttggtatcatgcctaaacagaaggggcgctataaagccctgtcttttgagccgacagaaaaaacatcagaaggattcgataagatgtactatgactacttcccagatgccgcaaaaatgattcctaagtgttccactcagctaaaggctgtaaccgctcattttcaaactcataccacccccattcttctctcaaataatttcattgaacctcttgaaatcacaaaagaaatttatgacctgaacaatcctgaaaaggagcctaaaaagtttcaaacggcttatgcaaagaagacaggcgatcaaaaaggctatagagaagcgctttgcaaatggattgactttacgcgggattttctctctaaatatacgaaaacaacttcaatcgatttatcttcactccgcccttcttcgcaatataaagatttaggggaatattacgccgaactgaatccgcttctctatcatatctccttccaacgaattgctgaaaaggaaatcatggatgctgtagaaacgggaaaattgtatctgttccaaatctacaataaggattttgcgaagggccatcacgggaaaccaaatctccacaccctgtattggacaggtctcttcagtcctgaaaaccttgcgaaaaccagcatcaaacttaatggtcaagcagaattgttctatcgacctaaaagccgcatgaagcggatggcccatcgtcttggggaaaaaatgctgaacaaaaaactaaaggaccagaagacaccgattccagataccctctaccaagaactgtacgattatgtcaaccaccggctaagccatgatctttccgatgaagcaagggccctgcttccaaatgttatcaccaaagaagtctcccatgaaattataaaggatcggcggtttacttccgataaatttttcttccatgttcccattacactgaattatcaagcagccaatagtcccagtaaattcaaccagcgtgtcaatgcctaccttaaggagcatccggaaacgcccatcattggtatcgatcgtggagaacgcaatctaatctatattaccgtcattgacagtactgggaaaattttggagcagcgttccctgaataccatccagcaatttgactaccaaaaaaaattggacaacagggaaaaagagcgtgttgccgcccgtcaagcctggtccgtcgtcggaacgatcaaagaccttaaacaaggctacttgtcacaggtcatccatgaaattgtagacctgatgattcattaccaagctgttgtcgtccttgaaaacctcaacttcggatttaaatcaaaacggacaggcattgccgaaaaagcagtctaccaacaatttgaaaagatgctaatagataaactcaactgtttggttctcaaagattatcctgctgagaaagtgggaggcgtcttaaacccgtatcaacttacagatcagttcacgagctttgcaaaaatgggcacgcaaagcggcttccttttctatgtaccggccccttatacctcaaagattgatcccctgactggttttgtcgatccctttgtatggaagaccattaaaaatcatgaaagtcggaagcatttcctagaaggatttgatttcctgcattatgatgtcaaaacaggtgattttatcctccattttaaaatgaatcggaatctctctttccagagagggcttcctggcttcatgccagcttgggatattgttttcgaaaagaatgaaacccaatttgatgcaaaagggacgcccttcattgcaggaaaacgaattgttcctgtaatcgaaaatcatcgttttacgggtcgttacagagacctctatcccgctaatgaactcattgcccttctggaagaaaaaggcattgtctttagagacggaagtaatatattacccaaacttttagaaaatgatgattctcatgcaattgatacgatggtcgccttgattcgcagtgtactccaaatgagaaacagcaatgccgcaacgggggaagactacatcaactctcccgttagggatctgaacggggtgtgtttcgacagtcgattccaaaatccagaatggccaatggatgcggatgccaacggagcttatcatattgccttaaaagggcagcttcttctgaaccacctcaaagaaagcaaagatctgaaattacaaaacggcatcagcaaccaagattggctggcctacattcaggaactgagaaactga

SEQ ID NO: 2 - DNA, 189 bp, Solanum tuberosum
gtaagtttctgcttctacctttgatatatatataataattatcattaattagtagtaatataatatttcaaatatttttttcaaaataaaagaatgtagtatatagcaattgcttttctgtagtttataagtgtgtatattttaatttataacttttctaatatatgaccaaaacatggtgatgtgcag

SEQ ID NO: 3 - protein, 11 aa, Simian virus 40
SRADPKKKRKV

SEQ ID NO: 4 - DNA, 4146 bp, Artificial Sequence
  Maize Optimized Cpf1 Gene with Intron and NLS
atgacccagttcgagggcttcaccaacctctaccaggtcagcaagaccctcaggttcgagctcatcccccagggcaagaccctcaagcacatccaggagcaggtaagtttctgcttctacctttgatatatatataataattatcattaattagtagtaatataatatttcaaatatttttttcaaaataaaagaatgtagtatatagcaattgcttttctgtagtttataagtgtgtatattttaatttataacttttctaatatatgaccaaaacatggtgatgtgcagggcttcatcgaggaggacaaggcccgcaacgaccactacaaggagctcaaaccaatcatcgacaggatctacaagacctacgccgaccagtgcctccagctcgtccagctcgactgggagaacctcagcgccgccatcgactcataccgcaaggaaaagaccgaggagaccaggaacgccctcatcgaggagcaggccacctacaggaacgccatccacgactacttcatcggcaggaccgacaacctcaccgacgccataaataagcgccacgccgagatctacaagggcctcttcaaggccgagctcttcaacggcaaggtcctcaagcagctcggcaccgtcaccaccaccgagcatgaaaatgccctcctccgcagcttcgacaagttcaccacctacttcagcggcttctatgaaaaccgcaagaacgtgttcagcgccgaggacatcagcaccgccatcccccacaggatcgtccaggacaacttccccaagttcaaggagaactgccacatcttcacccgcctcatcaccgccgtccccagcctacgcgagcacttcgagaacgtcaagaaggccatcggcatcttcgtcagcaccagcatcgaggaggtgttcagcttccccttctacaatcaactcctcacccagacccagatcgacctctacaatcaactcctcggcggcatcagccgcgaggccggcaccgagaaaatcaagggcctcaacgaggtcctcaacctcgccatccagaagaacgatgaaacagcccatataatcgccagcctcccccacaggttcatcccgctcttcaagcagatcctcagcgaccgcaacaccctcagcttcatcctcgaggagttcaagagcgacgaggaggtcatccagagcttctgcaaatataaaaccctcctcaggaacgagaacgtcctcgagaccgccgaggccctcttcaacgaattaaatagcatcgacctcacccatatctttatcagccataaaaagctcgagactatcagcagcgccctctgcgaccactgggacaccctcaggaacgccctctacgagaggcgcatcagcgagctcaccggcaaaataaccaagagcgccaaggagaaggtccagcgctcattaaaacacgaggatataaatctccaggagatcatcagcgccgccggcaaggagctcagcgaagcattcaagcaaaagaccagcgagatcctcagccacgcccacgccgccctcgaccagcccctccccaccacattaaaaaagcaggaggagaaggagatcctcaagagccagctcgacagcctcctcggcctctaccacctgctcgactggttcgccgtcgatgaaagcaacgaggtcgaccccgagttcagcgcccgcctcaccggcattaaactcgagatggaaccaagcctcagcttctacaataaagcccgcaactacgccaccaagaagccctacagcgtcgagaagttcaagctcaacttccagatgcccaccctcgccagcggctgggacgtcaataaagagaaaaataatggcgccatcctcttcgtcaagaacggcctctactacctcggcatcatgcccaagcagaagggccgctacaaggccctcagcttcgagcccaccgaaaagaccagcgagggcttcgacaagatgtactacgactacttccccgacgccgccaagatgatccccaagtgcagcacccagctcaaggccgtcaccgcccacttccagacccacaccacccccatcctcctcagcaataatttcatcgagcccctcgagatcaccaaggagatctacgacctcaacaaccccgagaaggagcccaagaagttccagaccgcctacgccaaaaagaccggcgaccagaagggctacagggaggccctctgcaagtggatcgacttcacccgcgacttcctcagcaagtacaccaagaccaccagcatcgacctcagcagcctccgccccagctcccaatataaagacctcggcgagtactacgccgagctcaaccccctcctctaccacatcagcttccagcgcatcgccgagaaggagatcatggacgccgtcgagaccggcaagctctacctcttccagatctacaacaaggacttcgccaagggccaccacggcaaaccaaatctccacaccctctactggaccggcctcttcagccccgagaacctcgccaagaccagcatcaagctcaacggccaggccgagctattctacaggcccaagagcaggatgaagcgcatggcccaccgcctcggcgagaagatgctcaacaagaagctcaaggaccaaaagacccccatccccgacaccctctaccaggagctctacgactacgtcaaccacaggctcagccacgacctcagcgacgaggccagggccctcctcccgaacgtcatcaccaaggaggtcagccatgaaattatcaaggaccgccgcttcaccagcgacaagttcttcttccacgtccccatcaccctcaactaccaggccgccaacagccccagcaagttcaaccagcgcgtcaacgcctacctaaaggagcaccccgagacccccatcatcggcatcgaccgcggcgagcgcaacctcatctacatcaccgtcatcgacagcaccggcaagatcctcgagcagcgcagcctcaacaccatccagcagttcgactaccagaagaagctcgacaacagggagaaggagcgcgtcgccgccaggcaggcctggagcgtcgtcggcaccatcaaggacctcaagcagggctacctcagccaggtcatccatgaaattgtcgacctcatgatccactaccaggccgtcgtcgtcctcgagaacctcaacttcggcttcaaatcaaaacgcaccggcatcgccgagaaggccgtctaccagcagttcgagaagatgctcatcgacaagctcaactgcctcgtcctcaaggactaccccgccgagaaggtcggcggcgtcctcaacccctaccagctcaccgaccagttcaccagcttcgccaagatgggcacccagagcggcttcctcttctacgtccccgccccctacaccagcaagatcgaccccctcaccggcttcgtggaccccttcgtctggaaaaccattaaaaaccatgaaagtcgcaagcatttcctcgagggcttcgacttcctccactacgacgtcaagaccggcgacttcatcctccacttcaagatgaacaggaacctcagcttccagagggggctccccggcttcatgcccgcctgggacatcgtgttcgagaagaatgaaacccagttcgacgccaagggcacccccttcatcgccggcaagaggatcgtccccgtcatcgagaaccacaggttcaccggcaggtacagggacctctaccccgccaacgagctcatcgccctcctcgaggagaagggcatcgtgttccgcgacggcagcaacatcctccccaagctcctcgagaacgacgacagccacgccatcgacacgatggtcgccctcatcaggagcgtcctccagatgaggaacagcaacgccgccaccggcgaggactacatcaacagccccgtcagggacctcaacggcgtctgcttcgacagccgcttccagaaccccgagtggccgatggacgccgacgccaacggcgcctaccacatcgccctcaagggccagctcctcctcaaccacctcaaggagagcaaggacctcaagctccagaacggcatcagcaaccaagactggctcgcctacatccaggagctccgcaacagcagggccgacccgaagaagaagcgcaaggtgtag

SEQ ID NO: 5 - RNA, 20 nt, Acidaminococcus
uaauuucuacucuuguagau

SEQ ID NO: 6 - DNA, 1000 bp, Zea mays
tgagagtacaatgatgaacctagattaatcaatgccaaagtctgaaaaatgcaccctcagtctatgatccagaaaatcaagattgcttgaggccctgttcggttgttccggattagagccccggattaattcctagccggattacttctctaatttatatagattttgatgagctggaatgaatcctggcttattccggtacaaccgaacaggccctgaaggataccagtaatcgctgagctaaattggcatgctgtcagagtgtcagtattgcagcaaggtagtgagataaccggcatcatggtgccagtttgatggcaccattagggttagagatggtggccatgggcgcatgtcctggccaactttgtatgatatatggcagggtgaataggaaagtaaaattgtattgtaaaaagggatttcttctgtttgttagcgcatgtacaaggaatgcaagttttgagcgagggggcatcaaagatctggctgtgtttccagctgtttttgttagccccatcgaatccttgacataatgatcccgcttaaataagcaacctcgcttgtatagttccttgtgctctaacacacgatgatgataagtcgtaaaatagtggtgtccaaagaatttccaggcccagttgtaaaagctaaaatgctattcgaatttctactagcagtaagtcgtgtttagaaattatttttttatataccttttttccttctatgtacagtaggacacagtgtcagcgccgcgttgacggagaatatttgcaaaaaagtaaaagagaaagtcatagcggcgtatgtgccaaaaacttcgtcacagagagggccataagaaacatggcccacggcccaatacgaagcaccgcgacgaagcccaaacagcagtccgtaggtggagcaaagcgctgggtaatacgcaaacgttttgtcccaccttgactaatcacaagagtggagcgtaccttataaaccgagccgcaagcaccgaatt

SEQ ID NO: 7 - DNA, 27 bp, Zea mays
tttcattcatatggtgtccctgaccta

SEQ ID NO: 8 - DNA, 27 bp, Zea mays
tttactcttagctcatcacctatgtgg

SEQ ID NO: 9 - DNA, 27 bp, Zea mays
tttgggaacaccagccccttgagcacg

SEQ ID NO: 10 - protein, 1307 aa, Acidaminococcus
  MISC_FEATURE (1)..(1307): type V CRISPR-associated protein Cpf1 [Acidaminococcus sp. BV3L6]
  MISC_FEATURE (1)..(1307): gi545612232, type V CRISPR-associated protein Cpf1 [Acidaminococcus sp. BV3L6]
MTQFEGFTNLYQVSKTLRFELIPQGKTLKHIQEQGFIEEDKARNDHYKELKPIIDRIYKTYADQCLQLVQLDWENLSAAIDSYRKEKTEETRNALIEEQATYRNAIHDYFIGRTDNLTDAINKRHAEIYKGLFKAELFNGKVLKQLGTVTTTEHENALLRSFDKFTTYFSGFYENRKNVFSAEDISTAIPHRIVQDNFPKFKENCHIFTRLITAVPSLREHFENVKKAIGIFVSTSIEEVFSFPFYNQLLTQTQIDLYNQLLGGISREAGTEKIKGLNEVLNLAIQKNDETAHIIASLPHRFIPLFKQILSDRNTLSFILEEFKSDEEVIQSFCKYKTLLRNENVLETAEALFNELNSIDLTHIFISHKKLETISSALCDHWDTLRNALYERRISELTGKITKSAKEKVQRSLKHEDINLQEIISAAGKELSEAFKQKTSEILSHAHAALDQPLPTTLKKQEEKEILKSQLDSLLGLYHLLDWFAVDESNEVDPEFSARLTGIKLEMEPSLSFYNKARNYATKKPYSVEKFKLNFQMPTLASGWDVNKEKNNGAILFVKNGLYYLGIMPKQKGRYKALSFEPTEKTSEGFDKMYYDYFPDAAKMIPKCSTQLKAVTAHFQTHTTPILLSNNFIEPLEITKEIYDLNNPEKEPKKFQTAYAKKTGDQKGYREALCKWIDFTRDFLSKYTKTTSIDLSSLRPSSQYKDLGEYYAELNPLLYHISFQRIAEKEIMDAVETGKLYLFQIYNKDFAKGHHGKPNLHTLYWTGLFSPENLAKTSIKLNGQAELFYRPKSRMKRMAHRLGEKMLNKKLKDQKTPIPDTLYQELYDYVNHRLSHDLSDEARALLPNVITKEVSHEIIKDRRFTSDKFFFHVPITLNYQAANSPSKFNQRVNAYLKEHPETPIIGIDRGERNLIYITVIDSTGKILEQRSLNTIQQFDYQKKLDNREKERVAARQAWSVVGTIKDLKQGYLSQVIHEIVDLMIHYQAVVVLENLNFGFKSKRTGIAEKAVYQQFEKMLIDKLNCLVLKDYPAEKVGGVLNPYQLTDQFTSFAKMGTQSGFLFYVPAPYTSKIDPLTGFVDPFVWKTIKNHESRKHFLEGFDFLHYDVKTGDFILHFKMNRNLSFQRGLPGFMPAWDIVFEKNETQFDAKGTPFIAGKRIVPVIENHRFTGRYRDLYPANELIALLEEKGIVFRDGSNILPKLLENDDSHAIDTMVALIRSVLQMRNSNAATGEDYINSPVRDLNGVCFDSRFQNPEWPMDADANGAYHIALKGQLLLNHLKESKDLKLQNGISNQDWLAYIQELRN

SEQ ID NO: 11 - protein, 1318 aa, Artificial sequence
  maize optimized CPf1 with 3 prime NLS
MTQFEGFTNLYQVSKTLRFELIPQGKTLKHIQEQGFIEEDKARNDHYKELKPIIDRIYKTYADQCLQLVQLDWENLSAAIDSYRKEKTEETRNALIEEQATYRNAIHDYFIGRTDNLTDAINKRHAEIYKGLFKAELFNGKVLKQLGTVTTTEHENALLRSFDKFTTYFSGFYENRKNVFSAEDISTAIPHRIVQDNFPKFKENCHIFTRLITAVPSLREHFENVKKAIGIFVSTSIEEVFSFPFYNQLLTQTQIDLYNQLLGGISREAGTEKIKGLNEVLNLAIQKNDETAHIIASLPHRFIPLFKQILSDRNTLSFILEEFKSDEEVIQSFCKYKTLLRNENVLETAEALFNELNSIDLTHIFISHKKLETISSALCDHWDTLRNALYERRISELTGKITKSAKEKVQRSLKHEDINLQEIISAAGKELSEAFKQKTSEILSHAHAALDQPLPTTLKKQEEKEILKSQLDSLLGLYHLLDWFAVDESNEVDPEFSARLTGIKLEMEPSLSFYNKARNYATKKPYSVEKFKLNFQMPTLASGWDVNKEKNNGAILFVKNGLYYLGIMPKQKGRYKALSFEPTEKTSEGFDKMYYDYFPDAAKMIPKCSTQLKAVTAHFQTHTTPILLSNNFIEPLEITKEIYDLNNPEKEPKKFQTAYAKKTGDQKGYREALCKWIDFTRDFLSKYTKTTSIDLSSLRPSSQYKDLGEYYAELNPLLYHISFQRIAEKEIMDAVETGKLYLFQIYNKDFAKGHHGKPNLHTLYWTGLFSPENLAKTSIKLNGQAELFYRPKSRMKRMAHRLGEKMLNKKLKDQKTPIPDTLYQELYDYVNHRLSHDLSDEARALLPNVITKEVSHEIIKDRRFTSDKFFFHVPITLNYQAANSPSKFNQRVNAYLKEHPETPIIGIDRGERNLIYITVIDSTGKILEQRSLNTIQQFDYQKKLDNREKERVAARQAWSVVGTIKDLKQGYLSQVIHEIVDLMIHYQAVVVLENLNFGFKSKRTGIAEKAVYQQFEKMLIDKLNCLVLKDYPAEKVGGVLNPYQLTDQFTSFAKMGTQSGFLFYVPAPYTSKIDPLTGFVDPFVWKTIKNHESRKHFLEGFDFLHYDVKTGDFILHFKMNRNLSFQRGLPGFMPAWDIVFEKNETQFDAKGTPFIAGKRIVPVIENHRFTGRYRDLYPANELIALLEEKGIVFRDGSNILPKLLENDDSHAIDTMVALIRSVLQMRNSNAATGEDYINSPVRDLNGVCFDSRFQNPEWPMDADANGAYHIALKGQLLLNHLKESKDLKLQNGISNQDWLAYIQELRNSRADPKKKRKV

SEQ ID NO: 12 - DNA, 896 bp, Zea mays
gtgcagcgtgacccggtcgtgcccctctctagagataatgagcattgcatgtctaagttataaaaaattaccacatattttttttgtcacacttgtttgaagtgcagtttatctatctttatacatatatttaaactttactctacgaataatataatctatagtactacaataatatcagtgttttagagaatcatataaatgaacagttagacatggtctaaaggacaattgagtattttgacaacaggactctacagttttatctttttagtgtgcatgtgttctcctttttttttgcaaatagcttcacctatataatacttcatccattttattagtacatccatttagggtttagggttaatggtttttatagactaatttttttagtacatctattttattctattttagcctctaaattaagaaaactaaaactctattttagtttttttatttaataatttagatataaaatagaataaaataaagtgactaaaaattaaacaaataccctttaagaaattaaaaaaactaaggaaacatttttcttgtttcgagtagataatgccagcctgttaaacgccgtcgacgagtctaacggacaccaaccagcgaaccagcagcgtcgcgtcgggccaagcgaagcagacggcacggcatctctgtcgctgcctctggacccctctcgagagttccgctccaccgttggacttgctccgctgtcggcatccagaaattgcgtggcggagcggcagacgtgagccggcacggcaggcggcctcctcctcctctcacggcaccggcagctacgggggattcctttcccaccgctccttcgctttcccttcctcgcccgccgtaataaatagacaccccctccacaccctctt

SEQ ID NO: 13 - DNA, 82 bp, Zea mays
tccccaacctcgtgttgttcggagcgcacacacacacaaccagatctcccccaaatccacccgtcggcacctccgcttcaag

SEQ ID NO: 14 - DNA, 1013 bp, Zea mays
gtacgccgctcgtcctcccccccccccctctctaccttctctagatcggcgttccggtccatgcatggttagggcccggtagttctacttctgttcatgtttgtgttagatccgtgtttgtgttagatccgtgctgctagcgttcgtacacggatgcgacctgtacgtcagacacgttctgattgctaacttgccagtgtttctctttggggaatcctgggatggctctagccgttccgcagacgggatcgatttcatgattttttttgtttcgttgcatagggtttggtttgcccttttcctttatttcaatatatgccgtgcacttgtttgtcgggtcatcttttcatgcttttttttgtcttggttgtgatgatgtggtctggttgggcggtcgttctagatcggagtagaattctgtttcaaactacctggtggatttattaattttggatctgtatgtgtgtgccatacatattcatagttacgaattgaagatgatggatggaaatatcgatctaggataggtatacatgttgatgcgggttttactgatgcatatacagagatgctttttgttcgcttggttgtgatgatgtggtgtggttgggcggtcgttcattcgttctagatcggagtagaatactgtttcaaactacctggtgtatttattaattttggaactgtatgtgtgtgtcatacatcttcatagttacgagtttaagatggatggaaatatcgatctaggataggtatacatgttgatgtgggttttactgatgcatatacatgatggcatatgcagcatctattcatatgctctaaccttgagtacctatctattataataaacaagtatgttttataattattttgatcttgatatacttggatgatggcatatgcagcagctatatgtggatttttttagccctgccttcatacgctatttatttgcttggtactgtttcttttgtcgatgctcaccctgttgtttggtgttacttctgcag

SEQ ID NO: 15 - RNA, 44 nt, Artificial Sequence
  synthesized AsCpf1 Maize Optimized Guide RNA
  misc_feature (22)..(44): n is a, c, g, or u
guaauuucuacucuuguagaunnnnnnnnnnnnnnnnnnnnnnn

SEQ ID NO: 16 - RNA, 44 nt, Artificial Sequence
  synthesized Guide RNA for AsMS26-1
guaauuucuacucuuguagauauucauauggugucccugaccua

SEQ ID NO: 17 - RNA, 44 nt, Artificial Sequence
  synthesized Guide RNA for AsLIGULELESS-1
guaauuucuacucuuguagaucucuuagcucaucaccuaugugg

SEQ ID NO: 18 - RNA, 44 nt, Artificial Sequence
  synthesized Guide RNA for AsMS45-1
guaauuucuacucuuguagauggaacaccagccccuugagcacg

SEQ ID NO: 19 - DNA, 1054 bp, Bannana Streak Virus
gataaaaaggagttgatcataagaacagacagccaggccattgtagccttctacaagaagcaagcggatcacaagccttcaagaacgagatggcttatgttgattgattacattactgggctcggaatcaacgttaaatttgagcacattgacggaaaagaaaatgtcctagctgacactttatcaagattggtccaagttctaatcacaagggttcatcatccagcagagactcagctagttgaagccgtcatggaagtcctgagcaatccgaaaaaggaagccttggataaggtaaatcattttatctttctaacccaacaatggattgcagaacaaagaaaggagcatatggtgaacacactgctccagttggaagaacctcaactacactgcggctgcaaagatcacacaacaggagaaagaaggaacgccgttcttctccaaagtcacacctcagccaacccgtatagatggttctataagtgtgcacaagacagatgtcacacttggatttggaaggacatcctggaccagtatgctgaagattatgccgcttacaccaggattggacttgaggcacttagccttgaagactggttcgaagaaccagaacccgatccacctgacccagtggaccgccagaagatagaagatatcctggacctgcaagatgtcagcaatgacgattgaaagattcccaggatagccggcggacgtggtggacccagtctaggtgcgatgcttagtcacgcacgatgactctgtcggaaggcatctttactttcggcaaactttaataatactttaggaaaagtattgtacaagttaggtgcagaatcaataatgcacccagctttagtcttgtctactgaattattgtgtcggttgcattattggatgcctgcgtgcaccctaagcaatccccggctctcatctctataagaggagcctttgtattcagttgcaagcatgcaagtcacacactgcaagcttacttctgagcaaaaagagttttgagtgaaataaatttgaagttcccccttacatcttg

SEQ ID NO: 20 - DNA, 971 bp, Zea mays
ccctagctccctgcggctgttacgcggtcccccatcaatcttctgttcttgcggttgtagcctgtgtaacagtgctagagtatgtatgataaataggttttaagtctgcttacatgacattttttattgtggaagagacatataaaaattagagagagtggttctcatgcaacggcggacggcccggtgctaaaagagcttcaagacaaaataatgaaacaggaagagagtagatttatctaagagccaactttattatatgaatgtgtttattgttggctttagatgatatggtaaggagttagagctaataatagataggctctattattattattattaattaaactcgctctaaggaggaaagtgggaggaagggacgaggacgaagactactggaagcatcgtgcatggatgatggatgtggtgtctcttaatgtaggtggccggaggatgtacgtgttaattgcgcgataagcactcagatccaaccgcaaactacctccacactgacacactgatagagagaaagagagacctccgacgactgccgccgcagatgagccacgtacgtatacgacgtctgccggccggctcaggctgccgccatcaccctgctcgaaagtcgcgttaggcggcgccagctacataggagtatctagtctagccagttagtatactactactgcgctgatgatgaattaactctgcatagatactgtacttgcctccctccaacacccaaccacctcctgctcggctcttaataacttggacacggatcgatgccatccaaggaagaacacgacgacgacgacggaacatccaccatgcaagcttgcatccatacgccgatacgcgtgcatccatccatccaccattatttccattttccaccgatcacacgtacacaggcctatttaaggagcgacatcccactgcaactctcctcaccactcatcaccagctag

SEQ ID NO: 21 - DNA, 856 bp, Zea mays
gtaaggttcccttccctcctcccctcacacccctgttcgtgttccttcggatcggatctcagtggtgatgttagacgtccgcggctgcctacgtagtggcattgccgcccgaaaggtttgtttaggtggggtagatccgaaacaggccggatctggaccatgtccgcggcggggcggcgggacttgatcgcgtagctgtcgtgtgcatttctccctaccagtggcggaatcggcgatgtggacctaagggctaaggcttatctgctgccttgaccatttcgtcgctgacaaaaacaaagtgacaatcatgccgttctctgtttgtttatctggatcgttattacgctgtgaatcctgcgatatgtggctaagtgatttttcttctttttctgggggcagtttagcctttgacccagtcctaggtgtggtcactaggactgtgtagcatgatgagtgaggttgcagcaggctgattgctagtggacgtttttttccccaatttgttaggttttcacgctccaggttgtgcaagtaattttgctagtgattgtgtgatccatcttcaacgttgaaccttgtttttccccctaaaacccccaacaggaaatcttgccccgacttctattgcaaaaattgtaacgcttagcaccctgattgactcaattcctgtcactaggcatgctcggtcaaaagcagatgatttaccacttagaaactgccctgcccctgctttccacatagcatttcgaactttttgactactattgacacccccctaacttgccgaactatttctctcttcagctactatttacctagttataattacataaatgtttgtgtgtatcttgtgcag

SEQ ID NO: 22 - DNA, 91 bp, Zea mays
ctctagcaaagcacttgccatctaccgaccgccgcattccaaacagcccgacgagctagcagagcggcaggcacctccctcctcaaggaac

SEQ ID NO: 23 - DNA, 151 bp, Zea mays
ctgcaaggaaaagtgcaggcaatattcagtactcgagagaatctacattttactcttagctcatcagttatgtgggataggtgaaggcgtgaagcactccgagtcttcttggctattcaaagtttccttttcactttgctttccttttggt

SEQ ID NO: 24 - DNA, 151 bp, Zea mays
ctgcaaggaaaagtgcaggcaatattcagtactcgagagaatctacattttactcttagctcatcgcagacatgggataggtgaaggcgtgaagcactccgagtcttcttggctattcaaagtttccttttcactttgctttccttttggt

SEQ ID NO: 25 - DNA, 160 bp, Zea mays
ctgcaaggaaaagtgcaggcaatattcagtactcgagagaatctacattttactcttagctcatcagttatgtcgcagacatgggataggtgaaggcgtgaagcactccgagtcttcttggctattcaaagtttccttttcactttgctttccttttggt

SEQ ID NO: 26 - DNA, 22 bp, Zea mays
gccttcacctatcccacatagg

SEQ ID NO: 27 - DNA, 35 bp, unknown
  DNA from Acidominococcus species BV3L6
gtcaaaagacctttttaatttctactcttgtagat

SEQ ID NO: 28 - DNA, 1217 bp, Artificial Sequence
  Polymerase III Multiplex Transcriptional Cassette Example
tgagagtacaatgatgaacctagattaatcaatgccaaagtctgaaaaatgcaccctcagtctatgatccagaaaatcaagattgcttgaggccctgttcggttgttccggattagagccccggattaattcctagccggattacttctctaatttatatagattttgatgagctggaatgaatcctggcttattccggtacaaccgaacaggccctgaaggataccagtaatcgctgagctaaattggcatgctgtcagagtgtcagtattgcagcaaggtagtgagataaccggcatcatggtgccagtttgatggcaccattagggttagagatggtggccatgggcgcatgtcctggccaactttgtatgatatatggcagggtgaataggaaagtaaaattgtattgtaaaaagggatttcttctgtttgttagcgcatgtacaaggaatgcaagttttgagcgagggggcatcaaagatctggctgtgtttccagctgtttttgttagccccatcgaatccttgacataatgatcccgcttaaataagcaacctcgcttgtatagttccttgtgctctaacacacgatgatgataagtcgtaaaatagtggtgtccaaagaatttccaggcccagttgtaaaagctaaaatgctattcgaatttctactagcagtaagtcgtgtttagaaattatttttttatataccttttttccttctatgtacagtaggacacagtgtcagcgccgcgttgacggagaatatttgcaaaaaagtaaaagagaaagtcatagcggcgtatgtgccaaaaacttcgtcacagagagggccataagaaacatggcccacggcccaatacgaagcaccgcgacgaagcccaaacagcagtccgtaggtggagcaaagcgctgggtaatacgcaaacgttttgtcccaccttgactaatcacaagagtggagcgtaccttataaaccgagccgcaagcaccgaattgtcaaaagacctttttaatttctactcttgtagatattcatatggtgtccctgacctagtcaaaagacctttttaatttctactcttgtagatctcttagctcatcacctatgtgggtcaaaagacctttttaatttctactcttgtagatggaacaccagccccttgagcacggtcaaaagacctttttaatttctactcttgtagattttttttt

SEQ ID NO: 29 - DNA, 2555 bp, Artificial Sequence
  Polymerase II Multiplex Transcriptional Cassette Example
gtgcagcgtgacccggtcgtgcccctctctagagataatgagcattgcatgtctaagttataaaaaattaccacatattttttttgtcacacttgtttgaagtgcagtttatctatctttatacatatatttaaactttactctacgaataatataatctatagtactacaataatatcagtgttttagagaatcatataaatgaacagttagacatggtctaaaggacaattgagtattttgacaacaggactctacagttttatctttttagtgtgcatgtgttctcctttttttttgcaaatagcttcacctatataatacttcatccattttattagtacatccatttagggtttagggttaatggtttttatagactaatttttttagtacatctattttattctattttagcctctaaattaagaaaactaaaactctattttagtttttttatttaataatttagatataaaatagaataaaataaagtgactaaaaattaaacaaataccctttaagaaattaaaaaaactaaggaaacatttttcttgtttcgagtagataatgccagcctgttaaacgccgtcgacgagtctaacggacaccaaccagcgaaccagcagcgtcgcgtcgggccaagcgaagcagacggcacggcatctctgtcgctgcctctggacccctctcgagagttccgctccaccgttggacttgctccgctgtcggcatccagaaattgcgtggcggagcggcagacgtgagccggcacggcaggcggcctcctcctcctctcacggcaccggcagctacgggggattcctttcccaccgctccttcgctttcccttcctcgcccgccgtaataaatagacaccccctccacaccctctttccccaacctcgtgttgttcggagcgcacacacacacaaccagatctcccccaaatccacccgtcggcacctccgcttcaaggtacgccgctcgtcctcccccccccccctctctaccttctctagatcggcgttccggtccatgcatggttagggcccggtagttctacttctgttcatgtttgtgttagatccgtgtttgtgttagatccgtgctgctagcgttcgtacacggatgcgacctgtacgtcagacacgttctgattgctaacttgccagtgtttctctttggggaatcctgggatggctctagccgttccgcagacgggatcgatttcatgattttttttgtttcgttgcatagggtttggtttgcccttttcctttatttcaatatatgccgtgcacttgtttgtcgggtcatcttttcatgcttttttttgtcttggttgtgatgatgtggtctggttgggcggtcgttctagatcggagtagaattctgtttcaaactacctggtggatttattaattttggatctgtatgtgtgtgccatacatattcatagttacgaattgaagatgatggatggaaatatcgatctaggataggtatacatgttgatgcgggttttactgatgcatatacagagatgctttttgttcgcttggttgtgatgatgtggtgtggttgggcggtcgttcattcgttctagatcggagtagaatactgtttcaaactacctggtgtatttattaattttggaactgtatgtgtgtgtcatacatcttcatagttacgagtttaagatggatggaaatatcgatctaggataggtatacatgttgatgtgggttttactgatgcatatacatgatggcatatgcagcatctattcatatgctctaaccttgagtacctatctattataataaacaagtatgttttataattattttgatcttgatatacttggatgatggcatatgcagcagctatatgtggatttttttagccctgccttcatacgctatttatttgcttggtactgtttcttttgtcgatgctcaccctgttgtttggtgttacttctgcaggtcgactctagaggatccatggtcaaaagacctttttaatttctactcttgtagatattcatatggtgtccctgacctagtcaaaagacctttttaatttctactcttgtagatctcttagctcatcacctatgtgggtcaaaagacctttttaatttctactcttgtagatggaacaccagccccttgagcacggtcaaaagacctttttaatttctactcttgtagattaggtaccgttaacctagacttgtccatcttctggattggccaacttaattaatgtatgaaataaaaggatgcacacatagtgacatgctaatcactataatgtgggcatcaaagttgtgtgttatgtgtaattactagttatctgaataaaagagaaagagatcatccatatttcttatcctaaatgaatgtcacgtgtctttataattctttgatgaaccagatgcatttcattaaccaaatccatatacatataaatattaatcatatataattaatatcaattgggttagcaaaacaaatctagtctaggtgtgttttgcgaatgcggcc

SEQ ID NO: 30 - DNA, 3903 bp, Francisella novicida
atgtcaatttatcaagaatttgttaataaatatagtttaagtaaaactctaagatttgagttaatcccacagggtaaaacacttgaaaacataaaagcaagaggtttgattttagatgatgagaaaagagctaaagactacaaaaaggctaaacaaataattgataaatatcatcagttttttatagaggagatattaagttcggtttgtattagcgaagatttattacaaaactattctgatgtttattttaaacttaaaaagagtgatgatgataatctacaaaaagattttaaaagtgcaaaagatacgataaagaaacaaatatctgaatatataaaggactcagagaaatttaagaatttgtttaatcaaaaccttatcgatgctaaaaaagggcaagagtcagatttaattctatggctaaagcaatctaaggataatggtatagaactatttaaagccaatagtgatatcacagatatagatgaggcgttagaaataatcaaatcttttaaaggttggacaacttattttaagggttttcatgaaaatagaaaaaatgtttatagtagcaatgatattcctacatctattatttataggatagtagatgataatttgcctaaatttctagaaaataaagctaagtatgagagtttaaaagacaaagctccagaagctataaactatgaacaaattaaaaaagatttggcagaagagctaacctttgatattgactacaaaacatctgaagttaatcaaagagttttttcacttgatgaagtttttgagatagcaaactttaataattatctaaatcaaagtggtattactaaatttaatactattattggtggtaaatttgtaaatggtgaaaatacaaagagaaaaggtataaatgaatatataaatctatactcacagcaaataaatgataaaacactcaaaaaatataaaatgagtgttttatttaagcaaattttaagtgatacagaatctaaatcttttgtaattgataagttagaagatgatagtgatgtagttacaacgatgcaaagtttttatgagcaaatagcagcttttaaaacagtagaagaaaaatctattaaagaaacactatctttattatttgatgatttaaaagctcaaaaacttgatttgagtaaaatttattttaaaaatgataaatctcttactgatctatcacaacaagtttttgatgattatagtgttattggtacagcggtactagaatatataactcaacaaatagcacctaaaaatcttgataaccctagtaagaaagagcaagaattaatagccaaaaaaactgaaaaagcaaaatacttatctctagaaactataaagcttgccttagaagaatttaataagcatagagatatagataaacagtgtaggtttgaagaaatacttgcaaactttgcggctattccgatgatatttgatgaaatagctcaaaacaaagacaatttggcacagatatctatcaaatatcaaaatcaaggtaaaaaagacctacttcaagctagtgcggaagatgatgttaaagctatcaaggatcttttagatcaaactaataatctcttacataaactaaaaatatttcatattagtcagtcagaagataaggcaaatattttagacaaggatgagcatttttatctagtatttgaggagtgctactttgagctagcgaatatagtgcctctttataacaaaattagaaactatataactcaaaagccatatagtgatgagaaatttaagctcaattttgagaactcgactttggctaatggttgggataaaaataaagagcctgacaatacggcaattttatttatcaaagatgataaatattatctgggtgtgatgaataagaaaaataacaaaatatttgatgataaagctatcaaagaaaataaaggcgagggttataaaaaaattgtttataaacttttacctggcgcaaataaaatgttacctaaggttttcttttctgctaaatctataaaattttataatcctagtgaagatatacttagaataagaaatcattccacacatacaaaaaatggtagtcctcaaaaaggatatgaaaaatttgagtttaatattgaagattgccgaaaatttatagatttttataaacagtctataagtaagcatccggagtggaaagattttggatttagattttctgatactcaaagatataattctatagatgaattttatagagaagttgaaaatcaaggctacaaactaacttttgaaaatatatcagagagctatattgatagcgtagttaatcagggtaaattgtacctattccaaatctataataaagatttttcagcttatagcaaagggcgaccaaatctacatactttatattggaaagcgctgtttgatgagagaaatcttcaagatgtggtttataagctaaatggtgaggcagagcttttttatcgtaaacaatcaatacctaaaaaaatcactcacccagctaaagaggcaatagctaataaaaacaaagataatcctaaaaaagagagtgtttttgaatatgatttaatcaaagataaacgctttactgaagataagtttttctttcactgtcctattacaatcaattttaaatctagtggagctaataagtttaatgatgaaatcaatttattgctaaaagaaaaagcaaatgatgttcatatattaagtatagatagaggtgaaagacatttagcttactatactttggtagatggtaaaggcaatatcatcaaacaagatactttcaacatcattggtaatgatagaatgaaaacaaactaccatgataagcttgctgcaatagagaaagatagggattcagctaggaaagactggaaaaagataaataacatcaaagagatgaaagagggctatctatctcaggtagttcatgaaatagctaagctagttatagagtataatgctattgtggtttttgaggatttaaattttggatttaaaagagggcgtttcaaggtagagaagcaggtctatcaaaagttagaaaaaatgctaattgagaaactaaactatctagttttcaaagataatgagtttgataaaactgggggagtgcttagagcttatcagctaacagcaccttttgagacttttaaaaagatgggtaaacaaacaggtattatctactatgtaccagctggttttacttcaaaaatttgtcctgtaactggttttgtaaatcagttatatcctaagtatgaaagtgtcagcaaatctcaagagttctttagtaagtttgacaagatttgttataaccttgataagggctattttgagtttagttttgattataaaaactttggtgacaaggctgccaaaggcaagtggactatagctagctttgggagtagattgattaactttagaaattcagataaaaatcataattgggatactcgagaagtttatccaactaaagagttggagaaattgctaaaagattattctatcgaatatgggcatggcgaatgtatcaaagcagctatttgcggtgagagcgacaaaaagttttttgctaagctaactagtgtcctaaatactatcttacaaatgcgtaactcaaaaacaggtactgagttagattatctaatttcaccagtagcagatgtaaatggcaatttctttgattcgcgacaggcgccaaaaaatatgcctcaagatgctgatgccaatggtgcttatcatattgggctaaaaggtctgatgctactaggtaggatcaaaaataatcaagagggcaaaaaactcaatttggttatcaaaaatgaagagtattttgagttcgtgcagaataggaataactaa

SEQ ID NO: 31 - DNA, 3687 bp, Lachnospiraceae bacterium
atgtctaaattagagaagtttacaaattgttactctttgtcaaaaacacttcgttttaaggcgattcctgttggaaaaacccaagaaaatattgataataaaagattgcttgtcgaggatgaaaaacgtgcagaagattataagggggttaaaaaattacttgataggtattatttatcatttattaatgatgttcttcattccattaaactaaagaatttaaataattatatttcgttgtttagaaagaaaactcggacggaaaaagaaaacaaagaattagaaaatttagagataaatttacgtaaagaaatcgctaaggcttttaagggtaatgaaggttataaatctttatttaagaaggatattatcgagacgatattgcctgaatttcttgatgataaagatgaaattgctttggttaattcatttaatggatttacaacggcatttaccggtttttttgataatagggaaaatatgttttcggaagaagctaaatcaacctcaattgcttttcgttgtattaatgagaatttaacaagatatatatcaaatatggatatatttgaaaaagttgatgcaattttcgataagcatgaagtacaggaaataaaagaaaaaattctaaacagtgattatgatgttgaagatttcttcgaaggagaattttttaattttgttcttacgcaagaaggtatcgatgtttataacgctataattggtggctttgtgacagaatccggagaaaaaataaaaggattaaatgaatatattaatttatataatcagaaaactaagcaaaaattaccgaagtttaagcctttatataaacaggttttatcagatagagagtcactttctttttatggcgaaggttatacatctgatgaggaagttttagaagtatttagaaatactcttaataagaattcagaaatattttcttcaattaagaaattggaaaagttatttaaaaacttcgatgaatattcaagtgcaggaattttcgtaaaaaatggaccggctatttctacaatttctaaggatatatttggagagtggaatgtaattagagacaaatggaatgcggagtacgatgatatacatttaaaaaagaaggctgtagtaacagaaaaatatgaagatgacaggcgtaaatcattcaaaaaaataggaagtttttcattggagcagttgcaagaatacgctgatgctgatctatctgtggtagagaagttaaaagaaatcattatccaaaaagtggatgagatatataaagtttatggctcgtcagaaaaattgttcgatgctgattttgtactagaaaaatcgttaaaaaagaatgatgcagttgtagcaataatgaaagatttactagattctgtgaagtcttttgaaaattatataaaagccttttttggagagggaaaagaaacaaatcgagatgaatcattttatggtgattttgttttggcatatgacattcttttgaaagtggatcatatttatgatgcaatacgaaattatgtgacacaaaaaccgtattcgaaagataagtttaaattatattttcaaaacccgcaatttatggggggctgggataaggataaagagacagactatagggcaactatacttagatatggctcaaagtattacttggcgattatggataaaaaatatgctaagtgcttgcaaaaaatagataaggatgatgtaaatggaaactatgaaaaaataaattataagttgcttccaggacctaataagatgcttccaaaggtgttttttagtaagaagtggatggcttattataatccgtcggaagatattcaaaaaatatataaaaatggaacatttaaaaaaggagatatgtttaatttaaatgattgtcataaattaattgatttctttaaggattcaatcagtcggtatccgaaatggagtaacgcatatgattttaacttttctgagaccgagaaatataaggatatagcaggtttttacagagaggttgaagaacaaggatataaagtatcatttgaaagtgcgtctaaaaaagaagttgataaattggtagaagaaggaaaattatacatgttccaaatttataataaagacttttcggataaaagtcatggaacgccaaatcttcatacaatgtattttaagttgctgtttgatgaaaataatcatggtcaaattaggctttctggtggtgctgagctattcatgcgacgtgcaagtttgaaaaaggaagaattagttgtgcatcctgccaatagcccgatagcgaataaaaacccggataatccaaagaaaacgactacgttgtcatatgatgtatacaaggacaaaagattttcggaagatcagtatgagttgcatatacctattgcaataaataaatgccctaaaaatatatttaagataaatacagaggttagagtgctgctgaagcatgatgataatccttatgttataggaattgataggggggagagaaatttactttacattgtggtggttgatggtaagggtaatattgtggagcaatattcgctgaatgaaataattaataattttaatggaattagaattaagacggattaccattcacttttggataaaaaggagaaggaaagatttgaagctcgtcaaaattggacgtctatagaaaacattaaagaactaaaagccggatatattagtcaggttgttcataagatatgtgagttggtagaaaaatatgatgcggtaattgcacttgaagatttgaattctggttttaagaatagtcgagttaaagttgaaaagcaagtatatcagaaatttgaaaaaatgctgattgataaacttaactatatggtagataagaaatctaatccttgcgctacgggtggtgctctgaaaggctatcaaattactaacaagtttgagagttttaagtcgatgagtacacaaaatggttttattttttatattccggcgtggttgactagcaaaattgatccgtcaacaggatttgtaaatttgttgaaaacaaagtatacgagcattgcagattcaaagaaatttataagttcttttgacagaattatgtatgtacctgaagaagatttattcgagtttgcattagattataagaatttttctcggacagacgcggattatataaaaaaatggaaactctatagctatggtaacaggattagaatatttagaaatcctaaaaaaaataatgtatttgattgggaagaggtatgtcttacatcagcctataaggaactttttaataaatatgggattaattatcagcaaggagatatacgagctctcttatgtgaacagagtgataaggcattctatagctcttttatggcattaatgtcactcatgctgcaaatgagaaatagtataacaggtaggacggatgtagattttttgatttcaccagtaaaaaattctgacggtattttttatgattccagaaattatgaagctcaggaaaatgcaatattaccgaaaaatgcagatgctaatggggcttataatatcgcaagaaaagttttgtgggctataggtcagtttaaaaaggctgaagatgaaaaacttgataaggttaaaattgcaatatcaaataaggaatggctcgaatatgcgcaaacaagtgttaagcattga

SEQ ID NO: 32 - protein, 1300 aa, Francisella novicida
MSIYQEFVNKYSLSKTLRFELIPQGKTLENIKARGLILDDEKRAKDYKKAKQIIDKYHQFFIEEILSSVCISEDLLQNYSDVYFKLKKSDDDNLQKDFKSAKDTIKKQISEYIKDSEKFKNLFNQNLIDAKKGQESDLILWLKQSKDNGIELFKANSDITDIDEALEIIKSFKGWTTYFKGFHENRKNVYSSNDIPTSIIYRIVDDNLPKFLENKAKYESLKDKAPEAINYEQIKKDLAEELTFDIDYKTSEVNQRVFSLDEVFEIANFNNYLNQSGITKFNTIIGGKFVNGENTKRKGINEYINLYSQQINDKTLKKYKMSVLFKQILSDTESKSFVIDKLEDDSDVVTTMQSFYEQIAAFKTVEEKSIKETLSLLFDDLKAQKLDLSKIYFKNDKSLTDLSQQVFDDYSVIGTAVLEYITQQIAPKNLDNPSKKEQELIAKKTEKAKYLSLETIKLALEEFNKHRDIDKQCRFEEILANFAAIPMIFDEIAQNKDNLAQISIKYQNQGKKDLLQASAEDDVKAIKDLLDQTNNLLHKLKIFHISQSEDKANILDKDEHFYLVFEECYFELANIVPLYNKIRNYITQKPYSDEKFKLNFENSTLANGWDKNKEPDNTAILFIKDDKYYLGVMNKKNNKIFDDKAIKENKGEGYKKIVYKLLPGANKMLPKVFFSAKSIKFYNPSEDILRIRNHSTHTKNGSPQKGYEKFEFNIEDCRKFIDFYKQSISKHPEWKDFGFRFSDTQRYNSIDEFYREVENQGYKLTFENISESYIDSVVNQGKLYLFQIYNKDFSAYSKGRPNLHTLYWKALFDERNLQDVVYKLNGEAELFYRKQSIPKKITHPAKEAIANKNKDNPKKESVFEYDLIKDKRFTEDKFFFHCPITINFKSSGANKFNDEINLLLKEKANDVHILSIDRGERHLAYYTLVDGKGNIIKQDTFNIIGNDRMKTNYHDKLAAIEKDRDSARKDWKKINNIKEMKEGYLSQVVHEIAKLVIEYNAIVVFEDLNFGFKRGRFKVEKQVYQKLEKMLIEKLNYLVFKDNEFDKTGGVLRAYQLTAPFETFKKMGKQTGIIYYVPAGFTSKICPVTGFVNQLYPKYESVSKSQEFFSKFDKICYNLDKGYFEFSFDYKNFGDKAAKGKWTIASFGSRLINFRNSDKNHNWDTREVYPTKELEKLLKDYSIEYGHGECIKAAICGESDKKFFAKLTSVLNTILQMRNSKTGTELDYLISPVADVNGNFFDSRQAPKNMPQDADANGAYHIGLKGLMLLGRIKNNQEGKKLNLVIKNEEYFEFVQNRNN

SEQ ID NO: 33 - protein, 1228 aa, Lachnospiraceae bacterium
MSKLEKFTNCYSLSKTLRFKAIPVGKTQENIDNKRLLVEDEKRAEDYKGVKKLLDRYYLSFINDVLHSIKLKNLNNYISLFRKKTRTEKENKELENLEINLRKEIAKAFKGNEGYKSLFKKDIIETILPEFLDDKDEIALVNSFNGFTTAFTGFFDNRENMFSEEAKSTSIAFRCINENLTRYISNMDIFEKVDAIFDKHEVQEIKEKILNSDYDVEDFFEGEFFNFVLTQEGIDVYNAIIGGFVTESGEKIKGLNEYINLYNQKTKQKLPKFKPLYKQVLSDRESLSFYGEGYTSDEEVLEVFRNTLNKNSEIFSSIKKLEKLFKNFDEYSSAGIFVKNGPAISTISKDIFGEWNVIRDKWNAEYDDIHLKKKAVVTEKYEDDRRKSFKKIGSFSLEQLQEYADADLSVVEKLKEIIIQKVDEIYKVYGSSEKLFDADFVLEKSLKKNDAVVAIMKDLLDSVKSFENYIKAFFGEGKETNRDESFYGDFVLAYDILLKVDHIYDAIRNYVTQKPYSKDKFKLYFQNPQFMGGWDKDKETDYRATILRYGSKYYLAIMDKKYAKCLQKIDKDDVNGNYEKINYKLLPGPNKMLPKVFFSKKWMAYYNPSEDIQKIYKNGTFKKGDMFNLNDCHKLIDFFKDSISRYPKWSNAYDFNFSETEKYKDIAGFYREVEEQGYKVSFESASKKEVDKLVEEGKLYMFQIYNKDFSDKSHGTPNLHTMYFKLLFDENNHGQIRLSGGAELFMRRASLKKEELVVHPANSPIANKNPDNPKKTTTLSYDVYKDKRFSEDQYELHIPIAINKCPKNIFKINTEVRVLLKHDDNPYVIGIDRGERNLLYIVVVDGKGNIVEQYSLNEIINNFNGIRIKTDYHSLLDKKEKERFEARQNWTSIENIKELKAGYISQVVHKICELVEKYDAVIALEDLNSGFKNSRVKVEKQVYQKFEKMLIDKLNYMVDKKSNPCATGGALKGYQITNKFESFKSMSTQNGFIFYIPAWLTSKIDPSTGFVNLLKTKYTSIADSKKFISSFDRIMYVPEEDLFEFALDYKNFSRTDADYIKKWKLYSYGNRIRIFRNPKKNNVFDWEEVCLTSAYKELFNKYGINYQQGDIRALLCEQSDKAFYSSFMALMSLMLQMRNSITGRTDVDFLISPVKNSDGIFYDSRNYEAQENAILPKNADANGAYNIARKVLWAIGQFKKAEDEKLDKVKIAISNKEWLEYAQTSVKH

SEQ ID NO: 34 - DNA, 24 bp, Zea mays
gacttgttcgggagttaggtcagg

SEQ ID NO: 35 - DNA, 22 bp, Zea mays
ggtgtccatgtcgtgctcaagg

SEQ ID NO: 36 - DNA, 4125 bp, Artificial Sequence
  synthesized sequence of Maize Optimized Fransincella novicida U112 Cpf1 Gene with Intron and NLS
atgagcatctaccaggagttcgtcaataaatacagcctcagcaagaccctccgcttcgagctcatcccccagggcaagaccctcgagaacataaaagccaggggcctgatcctggacgatgagaagagggccaaggtaagtttctgcttctacctttgatatatatataataattatcattaattagtagtaatataatatttcaaatatttttttcaaaataaaagaatgtagtatatagcaattgcttttctgtagtttataagtgtgtatattttaatttataacttttctaatatatgaccaaaacatggtgatgtgcaggactacaagaaggccaagcaaataattgacaagtaccaccagttcttcatcgaggagatcctcagcagcgtctgcatcagcgaggacctcctccagaactacagcgacgtctacttcaagctcaagaagagcgacgacgataacctccagaaggacttcaagagcgcgaaggataccatcaagaagcagatcagcgagtatataaaggactcagagaagttcaagaacctcttcaatcaaaacctcatcgacgccaagaagggccaggagagcgatctgatcctgtggctcaagcagagcaaggacaacggcatcgagctcttcaaggccaacagcgacatcaccgacatcgacgaggccctcgaaataatcaagagcttcaagggctggaccacctacttcaagggcttccatgaaaatagaaagaacgtctacagcagcaacgacatccccaccagcatcatctacaggatcgtcgacgacaacctccccaagttcctcgaaaataaagccaagtacgagagcctcaaggacaaggcccccgaggccatcaactacgagcaaattaaaaaggacctcgccgaggagctcaccttcgacatcgactacaagaccagcgaggtcaatcaacgcgtgttcagcctcgacgaggtgttcgagatcgccaacttcaataattacctcaatcaaagcggcatcaccaagttcaatactatcatcggcggcaagttcgtcaacggcgaaaatacaaagcgcaagggcatcaacgagtatataaatctctacagccagcaaataaatgataaaacactcaaaaaatataaaatgagcgtcctcttcaagcagatcctcagcgacaccgagagcaagtccttcgtcatcgacaagctcgaggacgacagcgacgtcgtcaccaccatgcagagcttctacgagcagatcgccgccttcaagaccgtcgaggagaagagcattaaagaaaccctcagcctcctcttcgacgacctcaaggcccagaagctcgacctcagcaagatctacttcaagaacgacaagagcctcaccgacctcagccagcaggtgttcgacgactacagcgtcatcggcaccgccgtcctcgagtatataactcagcagatcgcccccaagaacctcgacaaccccagcaagaaggagcaggaattaatagccaaaaagaccgagaaggcaaaatacctcagcctcgaaaccatcaagctcgccctcgaggagttcaacaagcatcgcgacatcgacaagcagtgccgcttcgaggagatcctcgccaacttcgccgccatccccatgatcttcgatgaaatagcccagaacaaggacaacctcgcccagatcagcatcaagtaccagaatcaaggcaagaaggatctgctgcaggcgagcgcggaggacgacgtcaaggccatcaaggacctcctcgaccagaccaataatctcctccataaactcaaaatattccacatcagccagagcgaggacaaggccaacatcctcgacaaggacgagcacttctacctcgtgttcgaggagtgctacttcgagctcgccaacatcgtccccctctacaacaagatccgcaactatataactcagaagccctacagcgacgagaagttcaagctcaacttcgagaacagcaccctcgccaacggctgggataaaaataaagagcccgacaacaccgccatcctcttcatcaaggacgataagtactacctgggcgtgatgaacaagaaaaataacaaaatattcgacgacaaggccatcaaggaaaataaaggcgagggctataaaaaaatcgtctacaagctcctacccggcgccaataaaatgctccccaaggtgttcttcagcgccaagagcataaaattctacaaccccagcgaggacatcctccgcatccgcaaccactcgacgcacaccaagaacggcagcccccagaagggctatgaaaaattcgagttcaacatcgaggactgccgcaagttcatcgacttctacaagcagagcatcagcaagcatcccgagtggaaggacttcgggttcaggttctccgatacccagagatataatagcatcgacgagttctaccgcgaggtcgagaatcaaggctacaagctcaccttcgaaaatataagcgagagctacatcgacagcgtcgtcaaccagggcaagctctacctcttccagatctacaataaagacttcagcgcctacagcaagggccggcccaacctccacaccctctactggaaggccctcttcgacgagcgcaacctccaggatgtggtgtacaagctgaacggcgaggccgagctcttctaccgcaagcaatcaatacccaagaagatcacccaccccgccaaggaggccatcgccaataaaaacaaggacaaccccaagaaggagagcgtgttcgagtacgacttaatcaaagacaagcgcttcaccgaggacaagttcttcttccactgccccatcacaatcaatttcaagagcagcggcgccaacaagttcaacgatgaaatcaatctcctcctcaaggagaaggccaacgatgtgcacatcctcagcatcgaccgcggcgagcgccacctagcctactacaccctcgtcgacggcaagggcaacatcatcaagcaggacaccttcaacatcatcggcaacgaccgcatgaaaaccaactaccacgacaagctcgccgccatcgagaaggacagggacagcgccaggaaggactggaagaagatcaacaacatcaaggagatgaaagagggctacctcagccaggtcgtccatgaaatagccaagctcgtcatcgagtacaacgccatcgtcgtgttcgaggacctcaacttcggcttcaagcgcggccgcttcaaggtcgagaagcaggtctaccagaagctcgagaagatgctcatcgagaagctcaactacctcgtgttcaaggacaacgagttcgataaaactggcggcgtcctccgcgcctaccagctcaccgcccccttcgaaaccttcaagaagatgggcaagcagaccggcatcatctactacgtccccgccggcttcaccagcaagatctgccccgtcaccggcttcgtcaaccagctctaccccaagtatgaaagtgtcagcaagagccaggagttcttcagcaagttcgacaagatctgctacaacctcgacaagggctacttcgagttcagcttcgactataaaaacttcggcgacaaggccgccaagggcaagtggaccatcgccagcttcggcagcaggctcatcaacttccgcaacagcgataaaaatcacaactgggacacccgcgaggtctaccccaccaaggagctcgagaagctcctcaaggactacagcatcgagtacggccacggcgagtgcatcaaggccgccatctgcggcgagagcgacaagaagttcttcgccaagctcaccagcgtcctcaatactatcctccagatgcgcaacagcaagaccggcaccgagctcgactacctcatcagccccgtcgccgacgtcaacggcaacttcttcgacagccgccaggcccccaaaaatatgccccaggacgccgacgccaacggcgcctaccacatcggcctcaagggcctcatgctcctcggcaggatcaaaaataatcaagagggcaagaagctcaacctcgtcatcaagaacgaggagtacttcgagttcgtccagaaccgcaacaacagccgcgccgaccccaagaagaagcgcaaggtctag

SEQ ID NO: 37 - DNA, 3909 bp, Artificial Sequence
  synthesized sequence of Maize Optimized Lachnospiraceae bacterium ND2006 Cpf1 Gene with Intron and NLS
atgagcaagctcgagaagttcaccaactgctacagcctcagcaagaccctccgcttcaaggccatccccgtcggcaagacccaggaaaatattgacaataaaagactcctcgtcgaggatgaaaaacgcgccgaggtaagtttctgcttctacctttgatatatatataataattatcattaattagtagtaatataatatttcaaatatttttttcaaaataaaagaatgtagtatatagcaattgcttttctgtagtttataagtgtgtatattttaatttataacttttctaatatatgaccaaaacatggtgatgtgcaggactacaagggcgtcaagaagctcctcgaccgctactacctcagcttcattaatgacgtcctccacagcattaaactcaagaacctcaataattacatcagcctcttcaggaaaaagaccaggaccgagaaggagaacaaggagctcgagaacctcgagatcaacctcaggaaggagatcgccaaggccttcaagggcaacgagggctacaagagcctcttcaagaaggacatcatcgaaaccatcctccccgagttcctcgacgacaaggatgaaattgccctcgtcaacagcttcaacggcttcaccaccgccttcaccggcttcttcgacaaccgcgaaaatatgttcagcgaggaggccaaatcaaccagcatcgccttcaggtgcattaatgagaacctcacccgctacatcagcaacatggacatcttcgagaaggtcgacgccatcttcgacaagcatgaggtccaggaaataaaagagaagatcctcaacagcgactacgacgtcgaggacttcttcgagggcgagttcttcaacttcgtcctcacccaggagggcatcgacgtctacaacgccatcatcggcggcttcgtcaccgagagcggcgagaaaataaaaggattaaatgagtacattaatttatataatcaaaagaccaagcagaagctccccaagttcaagcccttatataaacaggtcctcagcgacagggagtccctctcgttctacggcgagggctatacatctgacgaggaggtcctcgaggtgttccgcaacaccctcaacaagaactccgagatcttcagctcaattaagaagctcgagaagctcttcaagaacttcgacgagtacagcagcgccggcatcttcgtcaagaacggccccgccatcagcaccatcagcaaggacatcttcggcgagtggaacgtcatccgcgacaagtggaacgccgagtacgacgacatacatctcaagaagaaggccgtcgtcaccgaaaaatatgaggacgaccgccgcaagagcttcaagaaaataggcagcttcagcctcgagcagctccaggagtacgccgacgccgacctcagcgtcgtcgagaagctcaaggagattattatccagaaggtcgacgagatatataaagtctacggcagcagcgagaagctcttcgacgccgacttcgtcctcgagaagagcctcaagaagaacgacgccgtcgtcgcaataatgaaagacctcctcgacagcgtcaagagcttcgagaactatataaaagccttcttcggcgagggcaaggaaaccaaccgcgacgagagcttctacggcgacttcgtcctcgcctacgacatcctcctcaaggtcgaccacatctacgacgccatccgcaactacgtcacccagaagccctacagcaaggacaagttcaagctctacttccagaacccccagttcatgggcggctgggacaaggacaaggaaaccgactaccgcgccaccatcctccgctacggcagcaagtactacctcgccatcatggataaaaaatatgccaagtgcctacagaaaatagacaaggacgacgtcaacggcaactatgaaaaaataaattacaagctcctccccggccccaacaagatgctccccaaggtgttcttcagcaagaagtggatggcctactacaaccccagcgaggacatccagaaaatatataaaaatggcaccttcaagaagggcgacatgttcaacctcaacgactgccataaattaattgacttcttcaaggacagcatcagccgctaccccaagtggagcaacgcctacgacttcaacttcagcgaaaccgagaaatataaggacatcgccggcttctaccgcgaggtcgaggagcagggatataaagtcagcttcgagagcgccagcaagaaggaggtcgacaagctcgtcgaggagggcaagttatacatgttccagatctacaataaagacttcagcgataaaagtcacggcacccccaacctccacaccatgtacttcaagctcctcttcgatgaaaataatcacggccagatcaggctcagcggcggcgccgagctcttcatgcgccgcgccagcctaaagaaggaggagctcgtcgtccaccccgccaacagccccatcgccaataaaaaccccgacaaccccaaaaagaccaccaccctcagctacgacgtctacaaggacaagaggttcagcgaggaccagtacgagctccacatccccatcgcaataaataaatgccccaaaaatatattcaagatcaatacagaggtccgcgtcctcctcaagcatgacgacaacccctacgtcatcggcatcgacaggggcgagcgcaacctcctctacatcgtcgtcgtcgacggcaagggcaacatcgtcgagcagtacagcctcaatgaaataattaataatttcaacggcatcagaattaagaccgactaccacagcctcctcgataaaaaggagaaggagaggttcgaggcccgccagaactggaccagcatcgagaacattaaagagctcaaggccggctacatcagccaggtcgtccacaagatctgcgagctcgtcgaaaaatatgacgccgtcatcgccctcgaggacctcaacagcggcttcaagaacagccgcgtcaaggtcgagaagcaggtctaccagaagttcgagaagatgctcatcgacaagctcaactacatggtcgacaagaagagcaacccctgcgccaccggcggcgccctcaagggctaccagatcaccaacaagttcgagagcttcaagagcatgagcacccagaacggcttcatcttctacatccccgcctggctcaccagcaagatcgaccccagcaccggcttcgtcaacctcctcaagaccaagtacaccagcatcgccgacagcaagaagttcatcagcagcttcgaccgcatcatgtacgtccccgaggaggacctcttcgagttcgccctcgactacaagaacttcagccgcaccgacgccgactatataaaaaagtggaagctctacagctacggcaacaggatccgcatcttccgcaaccccaagaaaaataatgtgttcgactgggaggaggtctgcctcaccagcgcctacaaggagctcttcaataaatacggcattaattaccagcagggcgacatcagggccctcctctgcgagcagagcgacaaggccttctacagcagcttcatggcattaatgagcctcatgctccagatgcgcaacagcatcaccggccgcaccgacgtcgacttcctcatcagccccgtcaagaacagcgacggcatcttctacgacagccgcaactacgaggcccaggagaacgccatcctccccaagaacgccgacgccaacggcgcctacaacatcgccaggaaggtcctctgggccatcggccagttcaagaaggccgaggatgaaaaactcgacaaggtcaagatcgccatcagcaacaaggagtggctcgagtacgcccagaccagcgtcaagcatagccgcgccgaccccaagaagaagcgcaaggtctag

SEQ ID NO: 38 - RNA, 20 nt, Fransincella novicida
uaauuucuacuguuguagau

SEQ ID NO: 39 - RNA, 21 nt, Lachnospiraceae bacterium
uaauuucuacuaaguguagau

SEQ ID NO: 40 - RNA, 44 nt, Artificial Sequence
  Synthesized Fn Cpf1 Maize Optimized Guide RNA
  misc_feature (22)..(44): n is a, c, g, or u
guaauuucuacuguuguagaunnnnnnnnnnnnnnnnnnnnnnn

SEQ ID NO: 41 - RNA, 45 nt, Artificial Sequence
  Synthesized Lb Cpf1 Maize Optimized Guide RNA
  misc_feature (23)..(45): n is a, c, g, or u
guaauuucuacuaaguguagaunnnnnnnnnnnnnnnnnnnnnnn

SEQ ID NO: 42 - RNA, 44 nt, Artificial Sequence
  Synthesized Fn Cpf1 Maize Optimized Guide RNA Containing AsMS26-1 Variable Targeting Domain
guaauuucuacuguuguagauauucauauggugucccugaccua

SEQ ID NO: 43 - RNA, 45 nt, Artificial Sequence
  Synthesized Lb Cpf1 Maize Optimized Guide RNA Containing AsMS26-1 Variable Targeting Domain
guaauuucuacuaaguguagauauucauauggugucccugaccua

SEQ ID NO: 44 - DNA, 43 bp, artificial sequence
  synthetic oligonulceotide comprising DNA and RNA nucleotides
  misc_feature (1)..(43): hybrid DNA-RNA oligonucleotide
taauuucuacucuuguagaucucuuagcucaucaccuaugugg

SEQ ID NO: 45 - DNA, 43 bp, artificial sequence
  synthetic oligonulceotide comprising DNA and RNA nucleotides
  misc_feature (1)..(43): hybrid DNA-RNA oligonucleotide
uaauuucuacucuuguagaucucuuagcucaucaccuaugugg

SEQ ID NO: 46 - DNA, 43 bp, artificial sequence
  synthetic oligonulceotide comprising DNA and RNA nucleotides
  misc_feature (1)..(43): hybrid DNA-RNA oligonucleotide
uaauuucuacuctuguagaucucuuagcucaucaccuaugugg

SEQ ID NO: 47 - DNA, 43 bp, artificial sequence; identical to SEQ ID NO: 45
  synthetic oligonulceotide comprising DNA and RNA nucleotides
  misc_feature (1)..(43): hybrid DNA-RNA oligonucleotide

SEQ ID NO: 48 - RNA, 100 nt, Artificial Sequence
  synthetic oligonucleotide
ggccgaggucgacuaccggcguuuuagagcuagaaauagcaaguuaaaauaaggcuaguccguuaucaacuugaaaaaguggcaccgagucggugcuuuu

SEQ ID NO: 49 - DNA, 23 bp, Zea mays
ggccgaggtcgactaccggccgg

SEQ ID NO: 50 - DNA, 23 bp, Artificial Sequence
  synthetic oligonucleotide
  misc_feature (1)..(23): n is a, c, g, or t
nnnnnnnnnnnnnnnnnnnnnnn